European Patent Application EP 4 631 960 A1, published October 15, 2025. Title: Peptides having an inhibitory activity on osteoclast differentiation and uses thereof. Applicant: CAREGEN CO., LTD. The sequence listing filed with the application follows.

SEQUENCE LISTING (18 sequences)

SEQ ID NO: 1 - protein, 8 aa, synthetic construct
EGSNSRTI

SEQ ID NO: 2 - protein, 10 aa, synthetic construct
IIAPTGYYGN

SEQ ID NO: 3 - DNA, 20 bp, synthetic construct
  source 1..20: mol_type = other DNA
cctggtgacgtgagactttc

SEQ ID NO: 4 - DNA, 20 bp, synthetic construct
  source 1..20: mol_type = other DNA
ggctgctttcatggctagta

SEQ ID NO: 5 - DNA, 20 bp, synthetic construct
  source 1..20: mol_type = other DNA
gccaatctgctgaaagagaa

SEQ ID NO: 6 - DNA, 20 bp, synthetic construct
  source 1..20: mol_type = other DNA
tcagcttcagggtaggtgaa

SEQ ID NO: 7 - DNA, 20 bp, synthetic construct
  source 1..20: mol_type = other DNA
aaatcactctttaagaacag

SEQ ID NO: 8 - DNA, 20 bp, synthetic construct
  source 1..20: mol_type = other DNA
ttattgaatagcagtgacag

SEQ ID NO: 9 - DNA, 20 bp, synthetic construct
  source 1..20: mol_type = other DNA
acagagaagctgggatcctt

SEQ ID NO: 10 - DNA, 20 bp, synthetic construct
  source 1..20: mol_type = other DNA
cagcctgagttcaaacccta

SEQ ID NO: 11 - DNA, 20 bp, synthetic construct
  source 1..20: mol_type = other DNA
gacccatctctgtgtccatc

SEQ ID NO: 12 - DNA, 20 bp, synthetic construct
  source 1..20: mol_type = other DNA
gaaaaatgccctgttgtgtc

SEQ ID NO: 13 - DNA, 20 bp, synthetic construct
  source 1..20: mol_type = other DNA
gcaaggaacccaaggagtcg

SEQ ID NO: 14 - DNA, 20 bp, synthetic construct
  source 1..20: mol_type = other DNA
cagttggcccagaaagaggg

SEQ ID NO: 15 - DNA, 20 bp, synthetic construct
  source 1..20: mol_type = other DNA
atggggccttgcaaaagaaa

SEQ ID NO: 16 - DNA, 20 bp, synthetic construct
  source 1..20: mol_type = other DNA
gctaacaaccgcaacccctc

SEQ ID NO: 17 - DNA, 20 bp, synthetic construct
  source 1..20: mol_type = other DNA
accacagtccatgccatcac

SEQ ID NO: 18 - DNA, 20 bp, synthetic construct
  source 1..20: mol_type = other DNA
tccaccaccctgttgctgta